European Patent Application EP 4 721 764 A1, published April 8, 2026. Title: 一种靶向LPA的dsRNA及其应用. Applicant: 上海拓界生物医药科技有限公司. Application CN. The sequence listing filed with the application follows.

SEQUENCE LISTING (56 sequences)

SEQ ID NO: 1 - RNA, 19 nt, synthetic construct
  source 1..19: mol_type = other RNA; note = TJR100373
gctccttattgttatacga

SEQ ID NO: 2 - RNA, 21 nt, Synthetic construct
  source 1..21: mol_type = other RNA; note = TJR100373
tcgtataacaataaggagctg

SEQ ID NO: 3 - RNA, 19 nt, synthetic construct
  source 1..19: mol_type = other RNA
  modified_base 1..19: mod_base = OTHER; note; note (original language) = 具有如表2中S0187所示的修饰
gctccttattgttatacga

SEQ ID NO: 4 - RNA, 19 nt, Synthetic construct
  source 1..19: mol_type = other RNA
  modified_base 1..19: mod_base = OTHER; note; note (original language) = 具有如表2中S0277所示的修饰
gctccttattgttatacga

SEQ ID NO: 5 - RNA, 19 nt, Synthetic construct
  source 1..19: mol_type = other RNA
  modified_base 1..19: mod_base = OTHER; note; note (original language) = 具有如表2中S0736所示的修饰
gctccttattgttatacga

SEQ ID NO: 6 - RNA, 19 nt, Synthetic construct
  source 1..19: mol_type = other RNA
  modified_base 1..19: mod_base = OTHER; note; note (original language) = 具有如表2中S0187-1所示的修饰
gctccttattgttatacga

SEQ ID NO: 7 - RNA, 19 nt, Synthetic construct
  source 1..19: mol_type = other RNA
  modified_base 1..19: mod_base = OTHER; note; note (original language) = 具有如表2中S0277-1所示的修饰
gctccttattgttatacga

SEQ ID NO: 8 - RNA, 21 nt, Synthetic construct
  source 1..21: mol_type = other RNA
  modified_base 1..21: mod_base = OTHER; note; note (original language) = 具有如表2中A0160所示的修饰
tcgtataacaataaggagctg

SEQ ID NO: 9 - RNA, 21 nt, synthetic construct
  source 1..21: mol_type = other RNA
  modified_base 1..21: mod_base = OTHER; note; note (original language) = 具有如表2中A0545所示的修饰
tcgtataacaataaggagctg

SEQ ID NO: 10 - RNA, 21 nt, Synthetic construct
  source 1..21: mol_type = other RNA
  modified_base 1..21: mod_base = OTHER; note; note (original language) = 具有如表2中A0546所示的修饰
tcgtataacaataaggagctg

SEQ ID NO: 11 - RNA, 21 nt, Synthetic construct
  source 1..21: mol_type = other RNA
  modified_base 1..21: mod_base = OTHER; note; note (original language) = 具有如表2中A0547所示的修饰
tcgtataacaataaggagctg

SEQ ID NO: 12 - RNA, 21 nt, synthetic construct
  source 1..21: mol_type = other RNA
  modified_base 1..21: mod_base = OTHER; note; note (original language) = 具有如表2中A0548所示的修饰
tcgtataacaataaggagctg

SEQ ID NO: 13 - RNA, 21 nt, synthetic construct
  source 1..21: mol_type = other RNA
  modified_base 1..21: mod_base = OTHER; note; note (original language) = 具有如表2中A0549所示的修饰
tcgtataacaataaggagctg

SEQ ID NO: 14 - RNA, 21 nt, synthetic construct
  source 1..21: mol_type = other RNA
  modified_base 1..21: mod_base = OTHER; note; note (original language) = 具有如表2中A0550所示的修饰
tcgtataacaataaggagctg

SEQ ID NO: 15 - RNA, 21 nt, synthetic construct
  source 1..21: mol_type = other RNA
  modified_base 1..21: mod_base = OTHER; note; note (original language) = 具有如表2中A0551所示的修饰
tcgtataacaataaggagctg

SEQ ID NO: 16 - RNA, 21 nt, synthetic construct
  source 1..21: mol_type = other RNA
  modified_base 1..21: mod_base = OTHER; note; note (original language) = 具有如表2中A0552所示的修饰
tcgtataacaataaggagctg

SEQ ID NO: 17 - RNA, 21 nt, synthetic construct
  source 1..21: mol_type = other RNA
  modified_base 1..21: mod_base = OTHER; note; note (original language) = 具有如表2中A0553所示的修饰
tcgtataacaataaggagctg

SEQ ID NO: 18 - RNA, 21 nt, synthetic construct
  source 1..21: mol_type = other RNA
  modified_base 1..21: mod_base = OTHER; note; note (original language) = 具有如表2中A0554所示的修饰
tcgtataacaataaggagctg

SEQ ID NO: 19 - RNA, 21 nt, synthetic construct
  source 1..21: mol_type = other RNA
  modified_base 1..21: mod_base = OTHER; note; note (original language) = 具有如表2中A0555所示的修饰
tcgtataacaataaggagctg

SEQ ID NO: 20 - RNA, 21 nt, synthetic construct
  source 1..21: mol_type = other RNA
  modified_base 1..21: mod_base = OTHER; note; note (original language) = 具有如表2中A0556所示的修饰
tcgtataacaataaggagctg

SEQ ID NO: 21 - RNA, 21 nt, synthetic construct
  source 1..21: mol_type = other RNA
  modified_base 1..21: mod_base = OTHER; note; note (original language) = 具有如表2中A0258所示的修饰
tcgtataacaataaggagctg

SEQ ID NO: 22 - RNA, 21 nt, synthetic construct
  source 1..21: mol_type = other RNA
  modified_base 1..21: mod_base = OTHER; note; note (original language) = 具有如表2中A0276所示的修饰
tcgtataacaataaggagctg

SEQ ID NO: 23 - RNA, 21 nt, synthetic construct
  source 1..21: mol_type = other RNA
  modified_base 1..21: mod_base = OTHER; note; note (original language) = 具有如表2中A0277所示的修饰
tcgtataacaataaggagctg

SEQ ID NO: 24 - RNA, 21 nt, synthetic construct
  source 1..21: mol_type = other RNA
  modified_base 1..21: mod_base = OTHER; note; note (original language) = 具有如表2中A0278所示的修饰
tcgtataacaataaggagctg

SEQ ID NO: 25 - RNA, 21 nt, synthetic construct
  source 1..21: mol_type = other RNA
  modified_base 1..21: mod_base = OTHER; note; note (original language) = 具有如表2中A0279所示的修饰
tcgtataacaataaggagctg

SEQ ID NO: 26 - RNA, 21 nt, synthetic construct
  source 1..21: mol_type = other RNA
  modified_base 1..21: mod_base = OTHER; note; note (original language) = 具有如表2中A0280所示的修饰
tcgtataacaataaggagctg

SEQ ID NO: 27 - RNA, 21 nt, synthetic construct
  source 1..21: mol_type = other RNA
  modified_base 1..21: mod_base = OTHER; note; note (original language) = 具有如表2中A0281所示的修饰
tcgtataacaataaggagctg

SEQ ID NO: 28 - RNA, 21 nt, synthetic construct
  source 1..21: mol_type = other RNA
  modified_base 1..21: mod_base = OTHER; note; note (original language) = 具有如表2中A0282所示的修饰
tcgtataacaataaggagctg

SEQ ID NO: 29 - RNA, 21 nt, synthetic construct
  source 1..21: mol_type = other RNA
  modified_base 1..21: mod_base = OTHER; note; note (original language) = 具有如表2中A0283所示的修饰
tcgtataacaataaggagctg

SEQ ID NO: 30 - RNA, 21 nt, synthetic construct
  source 1..21: mol_type = other RNA
  modified_base 1..21: mod_base = OTHER; note; note (original language) = 具有如表2中A0284所示的修饰
tcgtataacaataaggagctg

SEQ ID NO: 31 - RNA, 21 nt, synthetic construct
  source 1..21: mol_type = other RNA
  modified_base 1..21: mod_base = OTHER; note; note (original language) = 具有如表2中A0285所示的修饰
tcgtataacaataaggagctg

SEQ ID NO: 32 - RNA, 21 nt, synthetic construct
  source 1..21: mol_type = other RNA
  modified_base 1..21: mod_base = OTHER; note; note (original language) = 具有如表2中A0286所示的修饰
tcgtataacaataaggagctg

SEQ ID NO: 33 - RNA, 21 nt, synthetic construct
  source 1..21: mol_type = other RNA
  modified_base 1..21: mod_base = OTHER; note; note (original language) = 具有如表2中A0825所示的修饰
tcgtataacaataaggagctg

SEQ ID NO: 34 - RNA, 21 nt, synthetic construct
  source 1..21: mol_type = other RNA
  modified_base 1..21: mod_base = OTHER; note; note (original language) = 具有如表2中A0826所示的修饰
tcgtataacaataaggagctg

SEQ ID NO: 35 - RNA, 21 nt, synthetic construct
  source 1..21: mol_type = other RNA
  modified_base 1..21: mod_base = OTHER; note; note (original language) = 具有如表2中A0827所示的修饰
tcgtataacaataaggagctg

SEQ ID NO: 36 - RNA, 19 nt, synthetic construct
  source 1..19: mol_type = other RNA; note = TJR100374
ctccttattgttatacgag

SEQ ID NO: 37 - RNA, 21 nt, synthetic construct
  source 1..21: mol_type = other RNA; note = TJR100374
ctcgtataacaataaggagct

SEQ ID NO: 38 - RNA, 19 nt, synthetic construct
  source 1..19: mol_type = other RNA; note = TJR100375
tccttattgttatacgagg

SEQ ID NO: 39 - RNA, 21 nt, synthetic construct
  source 1..21: mol_type = other RNA; note = TJR100375
cctcgtataacaataaggagc

SEQ ID NO: 40 - RNA, 19 nt, synthetic construct
  source 1..19: mol_type = other RNA; note = TJR100376
agctccttattgttatacg

SEQ ID NO: 41 - RNA, 21 nt, synthetic construct
  source 1..21: mol_type = other RNA; note = TJR100376
cgtataacaataaggagctgc

SEQ ID NO: 42 - RNA, 19 nt, synthetic construct
  source 1..19: mol_type = other RNA; note = TJR100377
cagctccttattgttatac

SEQ ID NO: 43 - RNA, 21 nt, synthetic construct
  source 1..21: mol_type = other RNA; note = TJR100377
gtataacaataaggagctgcc

SEQ ID NO: 44 - RNA, 19 nt, synthetic construct
  source 1..19: mol_type = other RNA; note = TJR100378
gcgccttattgttatacga

SEQ ID NO: 45 - RNA, 21 nt, synthetic construct
  source 1..21: mol_type = other RNA; note = TJR100378
tcgtataacaataaggcgctg

SEQ ID NO: 46 - RNA, 19 nt, synthetic construct
  source 1..19: mol_type = other RNA; note = TJR100379
gcaccttattgttatacga

SEQ ID NO: 47 - RNA, 21 nt, synthetic construct
  source 1..21: mol_type = other RNA; note = TJR100379
tcgtataacaataaggtgctg

SEQ ID NO: 48 - RNA, 21 nt, synthetic construct
  source 1..21: mol_type = other RNA; note = TJR100380
cagccccttattgttatacga

SEQ ID NO: 49 - RNA, 21 nt, synthetic construct
  source 1..21: mol_type = other RNA; note = TJR100380
tcgtataacaataaggggctg

SEQ ID NO: 50 - RNA, 19 nt, synthetic construct
  source 1..19: mol_type = other RNA
  modified_base 1..19: mod_base = OTHER; note; note (original language) = 具有如表2中S1757所示的修饰
gctccttattgttatacga

SEQ ID NO: 51 - RNA, 21 nt, synthetic construct
  source 1..21: mol_type = other RNA
  modified_base 1..21: mod_base = OTHER; note; note (original language) = 具有如表2中A1764所示的修饰
tcgtataacaataaggagctg

SEQ ID NO: 52 - RNA, 21 nt, synthetic construct
  source 1..21: mol_type = other RNA
  modified_base 1..21: mod_base = OTHER; note; note (original language) = 具有如表2中TJR014640S所示的修饰
cagccccttattgttatacga

SEQ ID NO: 53 - RNA, 21 nt, synthetic construct
  source 1..21: mol_type = other RNA
  modified_base 1..21: mod_base = OTHER; note; note (original language) = 具有如表2中TJR014643A所示的修饰
tcgtataacaataaggggctg

SEQ ID NO: 54 - RNA, 18 nt, synthetic construct
  source 1..18: mol_type = other RNA; note; note (original language) = 引物
tggagggcctctggtttg

SEQ ID NO: 55 - RNA, 18 nt, synthetic construct
  source 1..18: mol_type = other RNA; note; note (original language) = 引物
ggcgtgcacagccaagac

SEQ ID NO: 56 - RNA, 21 nt, synthetic construct
  source 1..21: mol_type = other RNA
  modified_base 1..21: mod_base = OTHER; note; note (original language) = 具有如hLPA-P-MGB所示的修饰的探针序列
cattttacaaggagtcacttc